European Patent Specification EP 3 570 851 B1, published September 18, 2024. Title: ADOPTIVE TRANSFER OF PLASMACYTOID DENDRITIC CELLS TO PREVENT OR TREAT OCULAR DISEASES AND CONDITIONS. Applicant: Tufts Medical Center, Inc. The sequence listing filed with the application follows.

SEQUENCE LISTING (24 sequences)

SEQ ID NO: 1 - DNA, 20 bp, Artificial Sequence
  Synthetic Construct
gcccagcttcatcacagagt

SEQ ID NO: 2 - DNA, 20 bp, Artificial Sequence
  Synthetic Construct
tgttgaaagatgactggctg

SEQ ID NO: 3 - DNA, 15 bp, Artificial Sequence
  Synthetic Construct
tggccagcgttgcca

SEQ ID NO: 4 - DNA, 18 bp, Artificial Sequence
  Synthetic Construct
tctgcagcaccccctgaa

SEQ ID NO: 5 - DNA, 18 bp, Artificial Sequence
  Synthetic Construct
agcattcccttgacacag

SEQ ID NO: 6 - DNA, 18 bp, Artificial Sequence
  Synthetic Construct
ggtctacagtgatgttgc

SEQ ID NO: 7 - DNA, 20 bp, Artificial Sequence
  Synthetic Construct
gaacctgctcttctctgagt

SEQ ID NO: 8 - DNA, 18 bp, Artificial Sequence
  Synthetic Construct
agctgaggaggtacagtg

SEQ ID NO: 9 - DNA, 19 bp, Artificial Sequence
  Synthetic Construct
tgctgtcactgatgctgct

SEQ ID NO: 10 - DNA, 20 bp, Artificial Sequence
  Synthetic Construct
ggcttcgtctacagcgtctt

SEQ ID NO: 11 - DNA, 20 bp, Artificial Sequence
  Synthetic Construct
tacaggaagctgctggaagg

SEQ ID NO: 12 - DNA, 19 bp, Artificial Sequence
  Synthetic Construct
tgggtgtcaaccagaggaa

SEQ ID NO: 13 - DNA, 22 bp, Artificial Sequence
  Synthetic Construct
caaagccacaatgttccaccag

SEQ ID NO: 14 - DNA, 22 bp, Artificial Sequence
  Synthetic Construct
gatgtcgtcgtcagacctctcg

SEQ ID NO: 15 - DNA, 20 bp, Artificial Sequence
  Synthetic Construct
cccactaacatcaaatgggg

SEQ ID NO: 16 - DNA, 20 bp, Artificial Sequence
  Synthetic Construct
gatgatgacccttttggctc

SEQ ID NO: 17 - DNA, 23 bp, Artificial Sequence
  Synthetic Construct
tcaatgacctgcaaggctgtctg

SEQ ID NO: 18 - DNA, 24 bp, Artificial Sequence
  Synthetic Construct
ggcatcttcctgggtcaggggaaa

SEQ ID NO: 19 - DNA, 25 bp, Artificial Sequence
  Synthetic Construct
ggataccaactattgcttcagctcc

SEQ ID NO: 20 - DNA, 25 bp, Artificial Sequence
  Synthetic Construct
aggctccaaatataggggcagggtc

SEQ ID NO: 21 - DNA, 18 bp, Artificial Sequence
  Synthetic Construct
aacgcgacgcacatcaag

SEQ ID NO: 22 - DNA, 20 bp, Artificial Sequence
  Synthetic Construct
ctggtacgcgatcagaaagc

SEQ ID NO: 23 - DNA, 20 bp, Artificial Sequence
  Synthetic Construct
cccactaacatcaaatgggg

SEQ ID NO: 24 - DNA, 20 bp, Artificial Sequence
  Synthetic Construct
gatgatgacccttttggctc